European Patent Application EP 4 269 424 A1, published November 1, 2023. Title: Novel antiviral compounds and use thereof. Applicant: Ivarsson Ylva Nilsson Jakob Överby Wernstedt Anna. The sequence listing filed with the application follows.

SEQUENCE LISTING (10 sequences)

SEQ ID NO: 1 - protein, 36 aa, Artificial Sequence
  G3BPi WT
YGRKKRRQRRRLTFGDFDEHEVDALASGITFGDFDD

SEQ ID NO: 2 - protein, 36 aa, Artificial Sequence
  G3BPi ctrl
YGRKKRRQRRRLGAGDADEHEVDALASGIGAGDADD

SEQ ID NO: 3 - protein, 32 aa, Artificial Sequence
  G3BPi spacer
YGRKKRRQRRRLTFGDFDEHEASGITFGDFDD

SEQ ID NO: 4 - protein, 19 aa, Artificial Sequence
  G3BPi one
YGRKKRRQRRRLTFGDFDE

SEQ ID NO: 5 - protein, 36 aa, Artificial Sequence
  G3BPi Nmut
YGRKKRRQRRRLGAGDADEHEVDALASGITFGDFDD

SEQ ID NO: 6 - protein, 36 aa, Artificial Sequence
  G3BPi Cmut
YGRKKRRQRRRLTFGDFDEHEVDALASGIGAGDADD

SEQ ID NO: 7 - protein, 26 aa, Artificial Sequence
  G3BPi WT minus CP
LTFGDFDEHEVDALASGITFGDFDDW

SEQ ID NO: 8 - protein, 22 aa, Artificial Sequence
  G3BPi spacer minus CP
LTFGDFDEHEASGITFGDFDDW

SEQ ID NO: 9 - protein, 24 aa, Artificial Sequence
  G3BPi spacer2
LTFGDFDEHEALASGITFGDFDDW

SEQ ID NO: 10 - protein, 26 aa, Artificial Sequence
  G3BPi spacer3
LTFGDFTGSTGSTGSTGITFGDFDDW